European Patent Application EP 4 122 471 A1, published January 25, 2023. Title: Theraputic agent for subretinal hyperreflective material or retinal disease with subretinal hyperreflective material. Applicant: RIBOMIC INC. The sequence listing filed with the application follows.

SEQUENCE LISTING (12 sequences)

SEQ ID NO: 1 - RNA, 38 nt, Artificial Sequence
  FGF2 Aptamer
gggauacuagggcauuaauguuaccaguguagucucga

SEQ ID NO: 2 - RNA, 37 nt, Artificial Sequence
  FGF2 Aptamer
gggaaacuagggcguuaacgugaccaguguuucucga

SEQ ID NO: 3 - RNA, 36 nt, Artificial Sequence
  FGF2 Aptamer
gggauacuagggcauuaauguuaccaguguaguccc

SEQ ID NO: 4 - RNA, 34 nt, Artificial Sequence
  FGF2 Aptamer
ggauacuagggcauuaauguuaccaguguagucc

SEQ ID NO: 5 - RNA, 38 nt, Artificial Sequence
  FGF2 Aptamer
ggggauacuagggcauuaauguuaccaguguagucccc

SEQ ID NO: 6 - RNA, 37 nt, Artificial Sequence
  FGF2 Aptamer
agggauacuagggcauuaauguuaccaguguaguccc

SEQ ID NO: 7 - RNA, 35 nt, Artificial Sequence
  FGF2 Aptamer
gggaaacuagggcguuaacgugaccaguguuuccc

SEQ ID NO: 8 - RNA, 36 nt, Artificial Sequence
  FGF2 Aptamer
cggauacuagggcauuaauguuaccaguguaguccg

SEQ ID NO: 9 - RNA, 36 nt, Artificial Sequence
  FGF2 Aptamer
ccgauacuagggcauuaauguuaccaguguagucgg

SEQ ID NO: 10 - RNA, 36 nt, Artificial Sequence
  FGF2 Aptamer
gggauacuagggcguuaacguuaccaguguaguccc

SEQ ID NO: 11 - RNA, 36 nt, Artificial Sequence
  FGF2 Aptamer
gggauacuagggccuuaagguuaccaguguaguccc

SEQ ID NO: 12 - RNA, 36 nt, Artificial Sequence
  FGF2 Aptamer
gggauacuagggcauuuauguuaccaguguaguccc